European Patent Specification EP 4 051 678 B1, published March 4, 2026. Title: Small Molecule Inhibitors of KRAS G12C Mutant. Applicant: Merck Sharp & Dohme Corp. The sequence listing filed with the application follows.

SEQUENCE LISTING (1 sequence)

SEQ ID NO: 1 - protein, 183 aa, Artificial
  Synthetic Protein
  biotin (10)..(10)
GLNDIFEAQKIEWHETEYKLVVVGACGVGKSALTIQLIQNHFVDEYDPTIEDSYRKQVVIDGETSLLDILDTAGQEEYSAMRDQYMRTGEGFLLVFAINNTKSFEDIHHYREQIKRVKDSEDVPMVLVGNKSDLPSRTVDTKQAQDLARSYGIPFIETSAKTRQGVDDAFYTLVREIRKHKEK